European Patent Specification EP 3 250 591 B1, published November 12, 2025. Title: Human Antibodies to Ebola Virus Glycoprotein. Applicant: Regeneron Pharmaceuticals, Inc. The sequence listing filed with the application follows.

SEQUENCE LISTING (318 sequences)

SEQ ID NO: 1 - DNA, 342 bp, Artificial Sequence
  synthetic
cagctgcagctgcaggagtcgggcccaggactggtgaagccttcggagaccctgtccctcacctgcactgtctctggtggctccatcagcagtagtagttactactggggctggatccgccagcccccagggaaggggctggagtggattgggagtatctattatgatggggacacctactacaacccgtccctcaagagtcgagtcaccatatccgtagacacgtccaagaaccagttctccctgaggctgagctctgtgaccgccgcagacacggcagtgtattactgtgcgagacagtttgactactggggccagggaaccctggtcaccgtctcctca

SEQ ID NO: 2 - protein, 114 aa, Artificial Sequence
  synthetic
QLQLQESGPGLVKPSETLSLTCTVSGGSISSSSYYWGWIRQPPGKGLEWIGSIYYDGDTYYNPSLKSRVTISVDTSKNQFSLRLSSVTAADTAVYYCARQFDYWGQGTLVTVSS

SEQ ID NO: 3 - DNA, 30 bp, Artificial Sequence
  synthetic
ggtggctccatcagcagtagtagttactac

SEQ ID NO: 4 - protein, 10 aa, Artificial Sequence
  synthetic
GGSISSSSYY

SEQ ID NO: 5 - DNA, 21 bp, Artificial Sequence
  synthetic
atctattatgatggggacacc

SEQ ID NO: 6 - protein, 7 aa, Artificial Sequence
  synthetic
IYYDGDT

SEQ ID NO: 7 - DNA, 18 bp, Artificial Sequence
  synthetic
gcgagacagtttgactac

SEQ ID NO: 8 - protein, 6 aa, Artificial Sequence
  synthetic
ARQFDY

SEQ ID NO: 9 - DNA, 321 bp, Artificial Sequence
  synthetic
gaaatagtgatgacgcagtctccagccaccctgtctgtgtctccaggggaaagagccaccctctcctgcagggccagtcagagtgttagtagcaacttagcctggtaccagcagaaacctggccaggctcccaggctcctcatctatggtgcatccaccagggccactggtatcccagccaggttcagtggcagtgggtctgggacagagttcactctcaccatcagcagcctgcagtctgaagattttgcagtttattactgtcagcagtataaaaactggccgatcaccttcggccaagggacacgactggagattaaa

SEQ ID NO: 10 - protein, 107 aa, Artificial Sequence
  synthetic
EIVMTQSPATLSVSPGERATLSCRASQSVSSNLAWYQQKPGQAPRLLIYGASTRATGIPARFSGSGSGTEFTLTISSLQSEDFAVYYCQQYKNWPITFGQGTRLEIK

SEQ ID NO: 11 - DNA, 18 bp, Artificial Sequence
  synthetic
cagagtgttagtagcaac

SEQ ID NO: 12 - protein, 6 aa, Artificial Sequence
  synthetic
QSVSSN

SEQ ID NO: 13 - DNA, 9 bp, Artificial Sequence
  synthetic
ggtgcatcc

SEQ ID NO: 14 - protein, 3 aa, Artificial Sequence
  synthetic
GAS

SEQ ID NO: 15 - DNA, 27 bp, Artificial Sequence
  synthetic
cagcagtataaaaactggccgatcacc

SEQ ID NO: 16 - protein, 9 aa, Artificial Sequence
  synthetic
QQYKNWPIT

SEQ ID NO: 17 - DNA, 354 bp, Artificial Sequence
  synthetic
gaggtgcagctggtggagtctgggggaggcttggtacagcctggggggtccctgagactctcctgtgcagcctctggattcaccttcagtagctacgacatgcactgggtccgccaagctacaggaaaaggtctggagtgggtctcagctattggtactgctggtgacacatactatccaggctccgtgaagggccgattcaccatctccagagaaaatgccaaaaactccttgtatcttcaaatgaacagcctgagagccggggacacggctgtgtattactgtgcaagaacatggttcggggagctttactttgactactggggccagggaaccctggtcaccgtctcctca

SEQ ID NO: 18 - protein, 118 aa, Artificial Sequence
  synthetic
EVQLVESGGGLVQPGGSLRLSCAASGFTFSSYDMHWVRQATGKGLEWVSAIGTAGDTYYPGSVKGRFTISRENAKNSLYLQMNSLRAGDTAVYYCARTWFGELYFDYWGQGTLVTVSS

SEQ ID NO: 19 - DNA, 24 bp, Artificial Sequence
  synthetic
ggattcaccttcagtagctacgac

SEQ ID NO: 20 - protein, 8 aa, Artificial Sequence
  synthetic
GFTFSSYD

SEQ ID NO: 21 - DNA, 21 bp, Artificial Sequence
  synthetic
attggtactgctggtgacaca

SEQ ID NO: 22 - protein, 7 aa, Artificial Sequence
  synthetic
IGTAGDT

SEQ ID NO: 23 - DNA, 36 bp, Artificial Sequence
  synthetic
gcaagaacatggttcggggagctttactttgactac

SEQ ID NO: 24 - protein, 12 aa, Artificial Sequence
  synthetic
ARTWFGELYFDY

SEQ ID NO: 25 - DNA, 339 bp, Artificial Sequence
  synthetic
gacatcgtgatgacccagtctccagactccctggctgtgtctctgggcgagagggccaccatcaactgcaagtccagccagagtgttttatacagctccaacaataagaactacttagcttggtaccagcagaaaccaggacagcctcctaagctgctcatttactgggcatctacccgggaatccggggtccctgaccgattcagtggcagcgggtctgggacagaattcactctcaccatcaccagcctgcaggctgaagatgtggcagtttattactgtcagcaatattatagtagtccgctcactttcggcggagggaccaaggtggagatcaaa

SEQ ID NO: 26 - protein, 113 aa, Artificial Sequence
  synthetic
DIVMTQSPDSLAVSLGERATINCKSSQSVLYSSNNKNYLAWYQQKPGQPPKLLIYWASTRESGVPDRFSGSGSGTEFTLTITSLQAEDVAVYYCQQYYSSPLTFGGGTKVEIK

SEQ ID NO: 27 - DNA, 36 bp, Artificial Sequence
  synthetic
cagagtgttttatacagctccaacaataagaactac

SEQ ID NO: 28 - protein, 12 aa, Artificial Sequence
  synthetic
QSVLYSSNNKNY

SEQ ID NO: 29 - DNA, 9 bp, Artificial Sequence
  synthetic
tgggcatct

SEQ ID NO: 30 - protein, 3 aa, Artificial Sequence
  synthetic
WAS

SEQ ID NO: 31 - DNA, 27 bp, Artificial Sequence
  synthetic
cagcaatattatagtagtccgctcact

SEQ ID NO: 32 - protein, 9 aa, Artificial Sequence
  synthetic
QQYYSSPLT

SEQ ID NO: 33 - DNA, 375 bp, Artificial Sequence
  synthetic
gaggtgcagctggtggagtctgggggaggcttggtacagcctggggggtccctgagactctcctgtgcagcctctggattcacctttagcagctatgccatgacctgggtccgccaggctccagggaagggcctggagtgggtctcaagtattagtggtagtggtactagcacatactacgcagactccgtgaagggccggttcaccatctccagagacaattccaagaacacactgtatctgcaaatgaacagcctgcgagccgaggacacggccctatattactgttcgagagatatatatacctggaacttcctctcactaattggcggtatggacgtctggggccaagggaccacggtcaccgtctcctca

SEQ ID NO: 34 - protein, 125 aa, Artificial Sequence
  synthetic
EVQLVESGGGLVQPGGSLRLSCAASGFTFSSYAMTWVRQAPGKGLEWVSSISGSGTSTYYADSVKGRFTISRDNSKNTLYLQMNSLRAEDTALYYCSRDIYTWNFLSLIGGMDVWGQGTTVTVSS

SEQ ID NO: 35 - DNA, 24 bp, Artificial Sequence
  synthetic
ggattcacctttagcagctatgcc

SEQ ID NO: 36 - protein, 8 aa, Artificial Sequence
  synthetic
GFTFSSYA

SEQ ID NO: 37 - DNA, 24 bp, Artificial Sequence
  synthetic
attagtggtagtggtactagcaca

SEQ ID NO: 38 - protein, 8 aa, Artificial Sequence
  synthetic
ISGSGTST

SEQ ID NO: 39 - DNA, 54 bp, Artificial Sequence
  synthetic
tcgagagatatatatacctggaacttcctctcactaattggcggtatggacgtc

SEQ ID NO: 40 - protein, 18 aa, Artificial Sequence
  synthetic
SRDIYTWNFLSLIGGMDV

SEQ ID NO: 41 - DNA, 321 bp, Artificial Sequence
  synthetic
gacatccagatgacccagtctccatcctccctgtctgcatctgtaggagacagagtcaccatcacttgccgggcaagtcagggcattagaattgatttaggctggtatcagcagaaaccagggaaagcccctaaccgcctgatctatgctgcatccagtttgcaaggtggggtcccatcaaggttcagcggcagtggatctgggacagaattcactctcacaatcagcagcctgcagcctgaagattttgcaacttattactgtctacagcaaaatagttacccgtggacgttcggccaagggaccaaggtggaaatcaaa

SEQ ID NO: 42 - protein, 107 aa, Artificial Sequence
  synthetic
DIQMTQSPSSLSASVGDRVTITCRASQGIRIDLGWYQQKPGKAPNRLIYAASSLQGGVPSRFSGSGSGTEFTLTISSLQPEDFATYYCLQQNSYPWTFGQGTKVEIK

SEQ ID NO: 43 - DNA, 18 bp, Artificial Sequence
  synthetic
cagggcattagaattgat

SEQ ID NO: 44 - protein, 6 aa, Artificial Sequence
  synthetic
QGIRID

SEQ ID NO: 45 - DNA, 9 bp, Artificial Sequence
  synthetic
gctgcatcc

SEQ ID NO: 46 - protein, 3 aa, Artificial Sequence
  synthetic
AAS

SEQ ID NO: 47 - DNA, 27 bp, Artificial Sequence
  synthetic
ctacagcaaaatagttacccgtggacg

SEQ ID NO: 48 - protein, 9 aa, Artificial Sequence
  synthetic
LQQNSYPWT

SEQ ID NO: 49 - DNA, 387 bp, Artificial Sequence
  synthetic
gaggtgcagctggtggagtctgggggaggcttggtacagcctggggggtccctgagactctcctgtgcagcctctggattcacctttagcagctatgccatgaactgggtccgccaggctccagggaaggggctggagtgggtctcagttattagtggtagtggtggttggagaaactacgcagactccgtgaagggccggatcaccatctccagagacaattccaagaacacgctgtatctgcaaatgaacaacctgagagccgaggacacggccgtatattattgtgcgaaagatcggggtgcgacttttggagtggttattttgggacccccctattacggtatggacgtctggggccaagggaccacggtcaccgtctcctca

SEQ ID NO: 50 - protein, 129 aa, Artificial Sequence
  synthetic
EVQLVESGGGLVQPGGSLRLSCAASGFTFSSYAMNWVRQAPGKGLEWVSVISGSGGWRNYADSVKGRITISRDNSKNTLYLQMNNLRAEDTAVYYCAKDRGATFGVVILGPPYYGMDVWGQGTTVTVSS

SEQ ID NO: 51 - DNA, 24 bp, Artificial Sequence
  synthetic
ggattcacctttagcagctatgcc

SEQ ID NO: 52 - protein, 8 aa, Artificial Sequence
  synthetic
GFTFSSYA

SEQ ID NO: 53 - DNA, 24 bp, Artificial Sequence
  synthetic
attagtggtagtggtggttggaga

SEQ ID NO: 54 - protein, 8 aa, Artificial Sequence
  synthetic
ISGSGGWR

SEQ ID NO: 55 - DNA, 66 bp, Artificial Sequence
  synthetic
gcgaaagatcggggtgcgacttttggagtggttattttgggacccccctattacggtatggacgtc

SEQ ID NO: 56 - protein, 22 aa, Artificial Sequence
  synthetic
AKDRGATFGVVILGPPYYGMDV

SEQ ID NO: 57 - DNA, 321 bp, Artificial Sequence
  synthetic
gacatccagatgacccagtctccatcctccctgtctgcatctgtaagagacagagtcaccatcacttgccgggcaagtcagagcattagcacttatttaaattggtatcagcagaaaccagggaaagcccctaagctcctgatctatgctgcatccagtttgcaaagtggggtcccatcaaggttcagtggcagtggatctgggacaggtttcactctcaccatcagcagtctgcaacctgaagattttgcaacttactactgtcaacagagttacagtatcccgtacacttttggccaggggaccaagctggagatcaaa

SEQ ID NO: 58 - protein, 107 aa, Artificial Sequence
  synthetic
DIQMTQSPSSLSASVRDRVTITCRASQSISTYLNWYQQKPGKAPKLLIYAASSLQSGVPSRFSGSGSGTGFTLTISSLQPEDFATYYCQQSYSIPYTFGQGTKLEIK

SEQ ID NO: 59 - DNA, 18 bp, Artificial Sequence
  synthetic
cagagcattagcacttat

SEQ ID NO: 60 - protein, 6 aa, Artificial Sequence
  synthetic
QSISTY

SEQ ID NO: 61 - DNA, 9 bp, Artificial Sequence
  synthetic
gctgcatcc

SEQ ID NO: 62 - protein, 3 aa, Artificial Sequence
  synthetic
AAS

SEQ ID NO: 63 - DNA, 27 bp, Artificial Sequence
  synthetic
caacagagttacagtatcccgtacact

SEQ ID NO: 64 - protein, 9 aa, Artificial Sequence
  synthetic
QQSYSIPYT

SEQ ID NO: 65 - DNA, 354 bp, Artificial Sequence
  synthetic
gaggtgcagctggtggagtctgggggaggcttggtacagcctggggggtccctgagactctcctgtgcagcctctggattcacctctagcagctatgccatgaactgggtccgccaggctccagggaaggggctggagtgggtctcaacaattagtggtatgggtggtagcacatactacgcagactccgtgaagggccggttcaccatctccagagacaattccaagaacacgctgtatctgcaaatgaacagcctgagagccgaggacacggccgtatattactgtgcgaaaaggggatatccccattcttttgatatctggggccaagggacaatggtcaccgtctcttca

SEQ ID NO: 66 - protein, 118 aa, Artificial Sequence
  synthetic
EVQLVESGGGLVQPGGSLRLSCAASGFTSSSYAMNWVRQAPGKGLEWVSTISGMGGSTYYADSVKGRFTISRDNSKNTLYLQMNSLRAEDTAVYYCAKRGYPHSFDIWGQGTMVTVSS

SEQ ID NO: 67 - DNA, 24 bp, Artificial Sequence
  synthetic
ggattcacctctagcagctatgcc

SEQ ID NO: 68 - protein, 8 aa, Artificial Sequence
  synthetic
GFTSSSYA

SEQ ID NO: 69 - DNA, 24 bp, Artificial Sequence
  synthetic
attagtggtatgggtggtagcaca

SEQ ID NO: 70 - protein, 8 aa, Artificial Sequence
  synthetic
ISGMGGST

SEQ ID NO: 71 - DNA, 33 bp, Artificial Sequence
  synthetic
gcgaaaaggggatatccccattcttttgatatc

SEQ ID NO: 72 - protein, 11 aa, Artificial Sequence
  synthetic
AKRGYPHSFDI

SEQ ID NO: 73 - DNA, 318 bp, Artificial Sequence
  synthetic
gacatccagatgacccagtctccatcctccctgtctgcatctgtaggagacagagtcaccatcacttgccgggcaagtcagagcattagcagctttttaaattggtatcagcagaaaccagggaaagcccctaaactcctgatctatgctgcatccagtttgcaaagtggggtcccatcaaggttcagtggcagtggatctgggacagatttcactctcaccatcagcagtctgcaacctgaagattttgcaacttactactgtcaacagagttacagtaccctcaccttcggccaagggacacgactggagattaaa

SEQ ID NO: 74 - protein, 106 aa, Artificial Sequence
  synthetic
DIQMTQSPSSLSASVGDRVTITCRASQSISSFLNWYQQKPGKAPKLLIYAASSLQSGVPSRFSGSGSGTDFTLTISSLQPEDFATYYCQQSYSTLTFGQGTRLEIK

SEQ ID NO: 75 - DNA, 18 bp, Artificial Sequence
  synthetic
cagagcattagcagcttt

SEQ ID NO: 76 - protein, 6 aa, Artificial Sequence
  synthetic
QSISSF

SEQ ID NO: 77 - DNA, 9 bp, Artificial Sequence
  synthetic
gctgcatcc

SEQ ID NO: 78 - protein, 3 aa, Artificial Sequence
  synthetic
AAS

SEQ ID NO: 79 - DNA, 24 bp, Artificial Sequence
  synthetic
caacagagttacagtaccctcacc

SEQ ID NO: 80 - protein, 8 aa, Artificial Sequence
  synthetic
QQSYSTLT

SEQ ID NO: 81 - DNA, 354 bp, Artificial Sequence
  synthetic
gaggtgcagctggtggagtctgggggaggcttggtacagcctggggggtccctgagactctcctgtgcagcctctgaattcacctttagcagctatgccatgagctgggtccgccaggctccagggaaggggctggagtgggtctcagctattagtggtagtagtggtagcacatactacgcagactccgtgaagggccggttcaccatctccagagacaattccaaaaagacgctgtatctacaaatgaacagcctgagagtcgaggacacggccgtatattactgtgcgaaaggggggtacccccattcttttgatatctggggccatgggacaatggtcaccgtctcttca

SEQ ID NO: 82 - protein, 118 aa, Artificial Sequence
  synthetic
EVQLVESGGGLVQPGGSLRLSCAASEFTFSSYAMSWVRQAPGKGLEWVSAISGSSGSTYYADSVKGRFTISRDNSKKTLYLQMNSLRVEDTAVYYCAKGGYPHSFDIWGHGTMVTVSS

SEQ ID NO: 83 - DNA, 24 bp, Artificial Sequence
  synthetic
gaattcacctttagcagctatgcc

SEQ ID NO: 84 - protein, 8 aa, Artificial Sequence
  synthetic
EFTFSSYA

SEQ ID NO: 85 - DNA, 24 bp, Artificial Sequence
  synthetic
attagtggtagtagtggtagcaca

SEQ ID NO: 86 - protein, 8 aa, Artificial Sequence
  synthetic
ISGSSGST

SEQ ID NO: 87 - DNA, 33 bp, Artificial Sequence
  synthetic
gcgaaaggggggtacccccattcttttgatatc

SEQ ID NO: 88 - protein, 11 aa, Artificial Sequence
  synthetic
AKGGYPHSFDI

SEQ ID NO: 89 - DNA, 318 bp, Artificial Sequence
  synthetic
gacatccagatgacccagtctccatcctccctgtctgcatctgtaggagacagagtcaccatcacttgccgggcaagtcagagcattagcagctttttaaattggtatcagcagaaaccagggaaagcccctaaactcctgatctatgctgcatccagtttgcaaagtggggtcccatcaaggttcagtggcagtggatctgggacagatttcactctcaccatcagcagtctgcaacctgaagattttgcaacttactactgtcaacagagttacagttccatcaccttcggccaagggacacgactggagattaaa

SEQ ID NO: 90 - protein, 106 aa, Artificial Sequence
  synthetic
DIQMTQSPSSLSASVGDRVTITCRASQSISSFLNWYQQKPGKAPKLLIYAASSLQSGVPSRFSGSGSGTDFTLTISSLQPEDFATYYCQQSYSSITFGQGTRLEIK

SEQ ID NO: 91 - DNA, 18 bp, Artificial Sequence
  synthetic
cagagcattagcagcttt

SEQ ID NO: 92 - protein, 6 aa, Artificial Sequence
  synthetic
QSISSF

SEQ ID NO: 93 - DNA, 9 bp, Artificial Sequence
  synthetic
gctgcatcc

SEQ ID NO: 94 - protein, 3 aa, Artificial Sequence
  synthetic
AAS

SEQ ID NO: 95 - DNA, 24 bp, Artificial Sequence
  synthetic
caacagagttacagttccatcacc

SEQ ID NO: 96 - protein, 8 aa, Artificial Sequence
  synthetic
QQSYSSIT

SEQ ID NO: 97 - DNA, 375 bp, Artificial Sequence
  synthetic
caggtgcagctggtggagtctgggggaggcgtggtccagcctgggaggtccctgagactctcctgtgcagcgtctggattcaccttcagtagttatggcatccactgggtccgccaggctccaggcaagtggctggagtgggtggcatttatatggtttgatggaagtaataaatactatgcagactccgtgaagggccgattcaccatctccagagacgattccaagaacacgctgtatctgcaaatgaacagcctgagagccgaggacacggctgtttattactgtgcgagagatggagagatttttggagtgcttatttcctctgatgcttttgatatctggggccaagggacaatggtcaccgtctcttca

SEQ ID NO: 98 - protein, 125 aa, Artificial Sequence
  synthetic
QVQLVESGGGVVQPGRSLRLSCAASGFTFSSYGIHWVRQAPGKWLEWVAFIWFDGSNKYYADSVKGRFTISRDDSKNTLYLQMNSLRAEDTAVYYCARDGEIFGVLISSDAFDIWGQGTMVTVSS

SEQ ID NO: 99 - DNA, 24 bp, Artificial Sequence
  synthetic
ggattcaccttcagtagttatggc

SEQ ID NO: 100 - protein, 8 aa, Artificial Sequence
  synthetic
GFTFSSYG

SEQ ID NO: 101 - DNA, 24 bp, Artificial Sequence
  synthetic
atatggtttgatggaagtaataaa

SEQ ID NO: 102 - protein, 8 aa, Artificial Sequence
  synthetic
IWFDGSNK

SEQ ID NO: 103 - DNA, 54 bp, Artificial Sequence
  synthetic
gcgagagatggagagatttttggagtgcttatttcctctgatgcttttgatatc

SEQ ID NO: 104 - protein, 18 aa, Artificial Sequence
  synthetic
ARDGEIFGVLISSDAFDI

SEQ ID NO: 105 - DNA, 321 bp, Artificial Sequence
  synthetic
gacatccagatgacccagtctccatcctccctgtctgcatctgtaggagacagagtcaccatcacttgccgggcaagtcggggcattagaaatgatttaggctggtttcagcagaaaccagggaaagcccctaagcgcctgatctatgttgcatccaatttgcaaagtggggtcccatcaaggttcagcggcagtggatctgggacagaattcactctcacaatcagcagcctgcagcctgaagattttgcaacttattactgtctacagcataatagttacccgatcaccttcggccaagggacacgactggagattaaa

SEQ ID NO: 106 - protein, 107 aa, Artificial Sequence
  synthetic
DIQMTQSPSSLSASVGDRVTITCRASRGIRNDLGWFQQKPGKAPKRLIYVASNLQSGVPSRFSGSGSGTEFTLTISSLQPEDFATYYCLQHNSYPITFGQGTRLEIK

SEQ ID NO: 107 - DNA, 18 bp, Artificial Sequence
  synthetic
cggggcattagaaatgat

SEQ ID NO: 108 - protein, 6 aa, Artificial Sequence
  synthetic
RGIRND

SEQ ID NO: 109 - DNA, 9 bp, Artificial Sequence
  synthetic
gttgcatcc

SEQ ID NO: 110 - protein, 3 aa, Artificial Sequence
  synthetic
VAS

SEQ ID NO: 111 - DNA, 27 bp, Artificial Sequence
  synthetic
ctacagcataatagttacccgatcacc

SEQ ID NO: 112 - protein, 9 aa, Artificial Sequence
  synthetic
LQHNSYPIT

SEQ ID NO: 113 - DNA, 354 bp, Artificial Sequence
  synthetic
gaggtgcagctggtggagtctgggggaggcttggtacagcctggggggtccctgagactctcctgtgcagcctctggattcaccttcagaagctacgacatgcactgggtccgccaaggttcaggaaaaggtctggagtgggtctcagctattggtactgctggtgacacatactatttaggctccgtgaagggccgattcaccatctccagagaaaatgccaagaactccttgtatcttcaaatgaacagcctgagagccggggacacggctgtgtattactgtgcaagagcgtggttcggggacgtattcctggactactggggccagggaaccctggtcaccgtctcctca

SEQ ID NO: 114 - protein, 118 aa, Artificial Sequence
  synthetic
EVQLVESGGGLVQPGGSLRLSCAASGFTFRSYDMHWVRQGSGKGLEWVSAIGTAGDTYYLGSVKGRFTISRENAKNSLYLQMNSLRAGDTAVYYCARAWFGDVFLDYWGQGTLVTVSS

SEQ ID NO: 115 - DNA, 24 bp, Artificial Sequence
  synthetic
ggattcaccttcagaagctacgac

SEQ ID NO: 116 - protein, 8 aa, Artificial Sequence
  synthetic
GFTFRSYD

SEQ ID NO: 117 - DNA, 21 bp, Artificial Sequence
  synthetic
attggtactgctggtgacaca

SEQ ID NO: 118 - protein, 7 aa, Artificial Sequence
  synthetic
IGTAGDT

SEQ ID NO: 119 - DNA, 36 bp, Artificial Sequence
  synthetic
gcaagagcgtggttcggggacgtattcctggactac

SEQ ID NO: 120 - protein, 12 aa, Artificial Sequence
  synthetic
ARAWFGDVFLDY

SEQ ID NO: 121 - DNA, 318 bp, Artificial Sequence
  synthetic
gaaatagtgatgacgcagtctccagccaccctgtctgtgtctccaggggaaagagccaccctctcctgcagggccagtcagagtgttagcagcaacttagcctggtaccagcagaaacctggccaggctcccaggctcctcatatatggtgcatccaccagggccactggtatcccagccaggttcagtggcagtgggtctgggacagagttcactctcaccatcagcagcctgcagtctgaagattttgcaggctattactgtcagcagtataataacaggctgactttcggcggagggaccaaggtggagatcaaa

SEQ ID NO: 122 - protein, 106 aa, Artificial Sequence
  synthetic
EIVMTQSPATLSVSPGERATLSCRASQSVSSNLAWYQQKPGQAPRLLIYGASTRATGIPARFSGSGSGTEFTLTISSLQSEDFAGYYCQQYNNRLTFGGGTKVEIK

SEQ ID NO: 123 - DNA, 18 bp, Artificial Sequence
  synthetic
cagagtgttagcagcaac

SEQ ID NO: 124 - protein, 6 aa, Artificial Sequence
  synthetic
QSVSSN

SEQ ID NO: 125 - DNA, 9 bp, Artificial Sequence
  synthetic
ggtgcatcc

SEQ ID NO: 126 - protein, 3 aa, Artificial Sequence
  synthetic
GAS

SEQ ID NO: 127 - DNA, 24 bp, Artificial Sequence
  synthetic
cagcagtataataacaggctgact

SEQ ID NO: 128 - protein, 8 aa, Artificial Sequence
  synthetic
QQYNNRLT

SEQ ID NO: 129 - DNA, 381 bp, Artificial Sequence
  synthetic
gaggtgcagctggtggagtctgggggaggcttggtccagcctggagggtccctgagactctcctgtgcagcctctggattcaccttcagtgaccactacatggtctgggtccgccaggctccagggaaggggctggagtgggttggccgtactagaaacaaagctaatagttatagcacagaatatgccgcgtctgtgaaaggcagattcaccatctcaagagatgattcaaagaagtcactgtatctgcaaatgaacagcctgaaaaccgaggacacggccgtgtattactgtgctagagggggggaaacactatggttcggggagtccaactacggtatggacgtctggggccaagggaccacggtcaccgtctcctca

SEQ ID NO: 130 - protein, 127 aa, Artificial Sequence
  synthetic
EVQLVESGGGLVQPGGSLRLSCAASGFTFSDHYMVWVRQAPGKGLEWVGRTRNKANSYSTEYAASVKGRFTISRDDSKKSLYLQMNSLKTEDTAVYYCARGGETLWFGESNYGMDVWGQGTTVTVSS

SEQ ID NO: 131 - DNA, 24 bp, Artificial Sequence
  synthetic
ggattcaccttcagtgaccactac

SEQ ID NO: 132 - protein, 8 aa, Artificial Sequence
  synthetic
GFTFSDHY

SEQ ID NO: 133 - DNA, 30 bp, Artificial Sequence
  synthetic
actagaaacaaagctaatagttatagcaca

SEQ ID NO: 134 - protein, 10 aa, Artificial Sequence
  synthetic
TRNKANSYST

SEQ ID NO: 135 - DNA, 54 bp, Artificial Sequence
  synthetic
gctagagggggggaaacactatggttcggggagtccaactacggtatggacgtc

SEQ ID NO: 136 - protein, 18 aa, Artificial Sequence
  synthetic
ARGGETLWFGESNYGMDV

SEQ ID NO: 137 - DNA, 324 bp, Artificial Sequence
  synthetic
gaaattgtgttgacgcagtctccagacaccctgtctttgtctccaggggaaagagccaccctctcctgcagggccagtcagagtgttagcagcacctacttagcctggtaccagcagaaacctggccaggctcccagtctcctcatctatggtgcatccagcagggccactggcatcccagacaggttcagtggcagcgggtctgggacagacttcactctcaccatcagcagactggagcctgaagattttgcagtgtattactgtcagcagtatggtaggtcacctctcactttcggcggagggaccaaggtggagatcaaa

SEQ ID NO: 138 - protein, 108 aa, Artificial Sequence
  synthetic
EIVLTQSPDTLSLSPGERATLSCRASQSVSSTYLAWYQQKPGQAPSLLIYGASSRATGIPDRFSGSGSGTDFTLTISRLEPEDFAVYYCQQYGRSPLTFGGGTKVEIK

SEQ ID NO: 139 - DNA, 21 bp, Artificial Sequence
  synthetic
cagagtgttagcagcacctac

SEQ ID NO: 140 - protein, 7 aa, Artificial Sequence
  synthetic
QSVSSTY

SEQ ID NO: 141 - DNA, 9 bp, Artificial Sequence
  synthetic
ggtgcatcc

SEQ ID NO: 142 - protein, 3 aa, Artificial Sequence
  synthetic
GAS

SEQ ID NO: 143 - DNA, 27 bp, Artificial Sequence
  synthetic
cagcagtatggtaggtcacctctcact

SEQ ID NO: 144 - protein, 9 aa, Artificial Sequence
  synthetic
QQYGRSPLT

SEQ ID NO: 145 - DNA, 348 bp, Artificial Sequence
  synthetic
caggtgcagctggtggagtctgggggaggcgtggtccagcctgggaggtccctgagactctcctgtgcagcgtctggcttcaccttcaataactatggcatgcactgggtccgccaggctccaggcatggggctggagtgggtggcagttatatggcacgatggaagtgataaatactatgcagactccgtgaagggccgattcaccatctccagagacaattccaagaacacgctgtatctgcaaatgaacagcctgagagccgaggacacggctgtgtattactgtgcgagaaattggaacctctttgactactggggccagggaaccctggtcactgtctcctca

SEQ ID NO: 146 - protein, 116 aa, Artificial Sequence
  synthetic
QVQLVESGGGVVQPGRSLRLSCAASGFTFNNYGMHWVRQAPGMGLEWVAVIWHDGSDKYYADSVKGRFTISRDNSKNTLYLQMNSLRAEDTAVYYCARNWNLFDYWGQGTLVTVSS

SEQ ID NO: 147 - DNA, 24 bp, Artificial Sequence
  synthetic
ggcttcaccttcaataactatggc

SEQ ID NO: 148 - protein, 8 aa, Artificial Sequence
  synthetic
GFTFNNYG

SEQ ID NO: 149 - DNA, 24 bp, Artificial Sequence
  synthetic
atatggcacgatggaagtgataaa

SEQ ID NO: 150 - protein, 8 aa, Artificial Sequence
  synthetic
IWHDGSDK

SEQ ID NO: 151 - DNA, 27 bp, Artificial Sequence
  synthetic
gcgagaaattggaacctctttgactac

SEQ ID NO: 152 - protein, 9 aa, Artificial Sequence
  synthetic
ARNWNLFDY

SEQ ID NO: 153 - DNA, 324 bp, Artificial Sequence
  synthetic
gacatccagatgacccagtctccatcctccctgtctgcatctgtaggagacagaatcaccatcacttgccgggcaagtcagagcatcagcacctatttacattggtatcagcagaaaccagggaaagcccctaagctcctgatctatgctgcatccactttgcagagtggggtcccatcaaggttcagtggcagtggatctgggacagatttcactctcaccatcagcagtctgcaacctgaagattttgcaacttactactgtcaacagagtttcagtacccctccgataaacttcggccaagggaccaagctggagatcaaa

SEQ ID NO: 154 - protein, 108 aa, Artificial Sequence
  synthetic
DIQMTQSPSSLSASVGDRITITCRASQSISTYLHWYQQKPGKAPKLLIYAASTLQSGVPSRFSGSGSGTDFTLTISSLQPEDFATYYCQQSFSTPPINFGQGTKLEIK

SEQ ID NO: 155 - DNA, 18 bp, Artificial Sequence
  synthetic
cagagcatcagcacctat

SEQ ID NO: 156 - protein, 6 aa, Artificial Sequence
  synthetic
QSISTY

SEQ ID NO: 157 - DNA, 9 bp, Artificial Sequence
  synthetic
gctgcatcc

SEQ ID NO: 158 - protein, 3 aa, Artificial Sequence
  synthetic
AAS

SEQ ID NO: 159 - DNA, 30 bp, Artificial Sequence
  synthetic
caacagagtttcagtacccctccgataaac

SEQ ID NO: 160 - protein, 10 aa, Artificial Sequence
  synthetic
QQSFSTPPIN

SEQ ID NO: 161 - DNA, 384 bp, Artificial Sequence
  synthetic
gaggtgcagctggtggagtctgggggaggcttggtccagcctggggggtccctgagactctcctgtgcagcctctaaattcacctttgacacctttgccatgagctgggtccgccaggctccagggaaggggttggaatgggtctcatttattagtagttctggtggtcgcacagactatgtagactccgtgaagggccggttcaccatctccagagacaattccaagaacaccctgtatctgcaaatgaacagcctgcgagccgaggacacggccgtatattactgtgcgaaagaacggacgatttttggagtgcttattctgggccccgacaactacggtatggacgtctggggccaagggaccacggtcaccgtctcctca

SEQ ID NO: 162 - protein, 128 aa, Artificial Sequence
  synthetic
EVQLVESGGGLVQPGGSLRLSCAASKFTFDTFAMSWVRQAPGKGLEWVSFISSSGGRTDYVDSVKGRFTISRDNSKNTLYLQMNSLRAEDTAVYYCAKERTIFGVLILGPDNYGMDVWGQGTTVTVSS

SEQ ID NO: 163 - DNA, 24 bp, Artificial Sequence
  synthetic
aaattcacctttgacacctttgcc

SEQ ID NO: 164 - protein, 8 aa, Artificial Sequence
  synthetic
KFTFDTFA

SEQ ID NO: 165 - DNA, 24 bp, Artificial Sequence
  synthetic
attagtagttctggtggtcgcaca

SEQ ID NO: 166 - protein, 8 aa, Artificial Sequence
  synthetic
ISSSGGRT

SEQ ID NO: 167 - DNA, 63 bp, Artificial Sequence
  synthetic
gcgaaagaacggacgatttttggagtgcttattctgggccccgacaactacggtatggacgtc

SEQ ID NO: 168 - protein, 21 aa, Artificial Sequence
  synthetic
AKERTIFGVLILGPDNYGMDV

SEQ ID NO: 169 - DNA, 324 bp, Artificial Sequence
  synthetic
gacatccagatgacccagtctccatcctccctgtctgcatttgtaggagacagagtcaccatcacttgccgggcaagtcagagcattagcacctatttaaattggtatcagcaaaaaccagggaaagcccctaaactcctgatctatgctgcatccagtttgcaaagtggggtctcatcaaggttcagtggcagtggatctgggacagatttcactctcaccatcagcagtctgcaacctgaagattttgcaacttactactgtcaacagagttacagtgcccctccgatcaccttcggccaagggacacgactggagattaaa

SEQ ID NO: 170 - protein, 108 aa, Artificial Sequence
  synthetic
DIQMTQSPSSLSAFVGDRVTITCRASQSISTYLNWYQQKPGKAPKLLIYAASSLQSGVSSRFSGSGSGTDFTLTISSLQPEDFATYYCQQSYSAPPITFGQGTRLEIK

SEQ ID NO: 171 - DNA, 18 bp, Artificial Sequence
  synthetic
cagagcattagcacctat

SEQ ID NO: 172 - protein, 6 aa, Artificial Sequence
  synthetic
QSISTY

SEQ ID NO: 173 - DNA, 9 bp, Artificial Sequence
  synthetic
gctgcatcc

SEQ ID NO: 174 - protein, 3 aa, Artificial Sequence
  synthetic
AAS

SEQ ID NO: 175 - DNA, 30 bp, Artificial Sequence
  synthetic
caacagagttacagtgcccctccgatcacc

SEQ ID NO: 176 - protein, 10 aa, Artificial Sequence
  synthetic
QQSYSAPPIT

SEQ ID NO: 177 - DNA, 384 bp, Artificial Sequence
  synthetic
caggtacagctgcagcagtcaggtccaggactggtgaagccctcgcagaccctctcactcacctgtgccatctccggggacagtgtctctagcaacattcctgcttggaactggatcaggcagtccccttcgagaggccttgagtggctgggaaggacatactacaggtccaagtggtataatgattatgcagtatctgtgaaaagtcgaataaccatcaatccagacacatccaagaaccacttctccctgcagctgaactctgtgactcccgaggacacggctgtgtattactgtgcaagaggaagggtctatgacaggtcttctaggtacttctacgctatggacgtctggggccaagggaccacggtcaccgtctcctca

SEQ ID NO: 178 - protein, 128 aa, Artificial Sequence
  synthetic
QVQLQQSGPGLVKPSQTLSLTCAISGDSVSSNIPAWNWIRQSPSRGLEWLGRTYYRSKWYNDYAVSVKSRITINPDTSKNHFSLQLNSVTPEDTAVYYCARGRVYDRSSRYFYAMDVWGQGTTVTVSS

SEQ ID NO: 179 - DNA, 30 bp, Artificial Sequence
  synthetic
ggggacagtgtctctagcaacattcctgct

SEQ ID NO: 180 - protein, 10 aa, Artificial Sequence
  synthetic
GDSVSSNIPA

SEQ ID NO: 181 - DNA, 27 bp, Artificial Sequence
  synthetic
acatactacaggtccaagtggtataat

SEQ ID NO: 182 - protein, 9 aa, Artificial Sequence
  synthetic
TYYRSKWYN

SEQ ID NO: 183 - DNA, 54 bp, Artificial Sequence
  synthetic
gcaagaggaagggtctatgacaggtcttctaggtacttctacgctatggacgtc

SEQ ID NO: 184 - protein, 18 aa, Artificial Sequence
  synthetic
ARGRVYDRSSRYFYAMDV

SEQ ID NO: 185 - DNA, 324 bp, Artificial Sequence
  synthetic
gacatccagatgacccagtctccatcctccctgtctgcatctgtaggagacagagtcaccatcacttgccgggcaagtcagagcattagcagctatttaaattggtatcagcagaaaccagggaaagcccctaagctcctgatctatgctgcatccagtttgcaaagtggggtcccatcaaggttcagtggcagtggatctgggacagatttcactctcaccatcagcagtctgcaacctgaagattttgcaacttactactgtcaacagagttacagtaattatccgatcaccttcggccaagggacacgactggagattaaa

SEQ ID NO: 186 - protein, 108 aa, Artificial Sequence
  synthetic
DIQMTQSPSSLSASVGDRVTITCRASQSISSYLNWYQQKPGKAPKLLIYAASSLQSGVPSRFSGSGSGTDFTLTISSLQPEDFATYYCQQSYSNYPITFGQGTRLEIK

SEQ ID NO: 187 - DNA, 18 bp, Artificial Sequence
  synthetic
cagagcattagcagctat

SEQ ID NO: 188 - protein, 6 aa, Artificial Sequence
  synthetic
QSISSY

SEQ ID NO: 189 - DNA, 9 bp, Artificial Sequence
  synthetic
gctgcatcc

SEQ ID NO: 190 - protein, 3 aa, Artificial Sequence
  synthetic
AAS

SEQ ID NO: 191 - DNA, 30 bp, Artificial Sequence
  synthetic
caacagagttacagtaattatccgatcacc

SEQ ID NO: 192 - protein, 10 aa, Artificial Sequence
  synthetic
QQSYSNYPIT

SEQ ID NO: 193 - DNA, 357 bp, Artificial Sequence
  synthetic
gaggtgcagctggtggagtctgggggaggcttggttcagccgggggggtccctgagactctcctgtgcagcctctggattcaccttcagaacctacgacatgcactgggtccgccaagctacaggaaaaggtctggagtgggtctcagctattggtactgctggtgacacatactatccaggctccgtgaagggccgattcaccatctccagagaaaatgccaagaactccttgtatcttcaaatgaacagcctgagagccggtgacacggctgtgtattactgtgcacgaacgatttttggagtggttcttacctttgactactggggccagggaaccctggtcaccgtctcctca

SEQ ID NO: 194 - protein, 119 aa, Artificial Sequence
  synthetic
EVQLVESGGGLVQPGGSLRLSCAASGFTFRTYDMHWVRQATGKGLEWVSAIGTAGDTYYPGSVKGRFTISRENAKNSLYLQMNSLRAGDTAVYYCARTIFGVVLTFDYWGQGTLVTVSS

SEQ ID NO: 195 - DNA, 24 bp, Artificial Sequence
  synthetic
ggattcaccttcagaacctacgac

SEQ ID NO: 196 - protein, 8 aa, Artificial Sequence
  synthetic
GFTFRTYD

SEQ ID NO: 197 - DNA, 21 bp, Artificial Sequence
  synthetic
attggtactgctggtgacaca

SEQ ID NO: 198 - protein, 7 aa, Artificial Sequence
  synthetic
IGTAGDT

SEQ ID NO: 199 - DNA, 39 bp, Artificial Sequence
  synthetic
gcacgaacgatttttggagtggttcttacctttgactac

SEQ ID NO: 200 - protein, 13 aa, Artificial Sequence
  synthetic
ARTIFGVVLTFDY

SEQ ID NO: 201 - DNA, 324 bp, Artificial Sequence
  synthetic
gacatccagatgacccagtctccatcctccctgtctgcatctgtaggagacagagtcaccatcacttgccgggcaagtcagagcattagcagctctttaaattggtatcagcagaaaccagggaaagcccctaagctcctgatctatgctgcatccagtttgcacagtggggtcccatcaaggttcagtggcagtggatctgggacagatttcactctcaccatcagcagtctgcaacctgaagattttgcaacttactactgtcaacagacttacagtatccctccgaccaccttcggccaagggaccaaggtggaaatcaaa

SEQ ID NO: 202 - protein, 108 aa, Artificial Sequence
  synthetic
DIQMTQSPSSLSASVGDRVTITCRASQSISSSLNWYQQKPGKAPKLLIYAASSLHSGVPSRFSGSGSGTDFTLTISSLQPEDFATYYCQQTYSIPPTTFGQGTKVEIK

SEQ ID NO: 203 - DNA, 18 bp, Artificial Sequence
  synthetic
cagagcattagcagctct

SEQ ID NO: 204 - protein, 6 aa, Artificial Sequence
  synthetic
QSISSS

SEQ ID NO: 205 - DNA, 9 bp, Artificial Sequence
  synthetic
gctgcatcc

SEQ ID NO: 206 - protein, 3 aa, Artificial Sequence
  synthetic
AAS

SEQ ID NO: 207 - DNA, 30 bp, Artificial Sequence
  synthetic
caacagacttacagtatccctccgaccacc

SEQ ID NO: 208 - protein, 10 aa, Artificial Sequence
  synthetic
QQTYSIPPTT

SEQ ID NO: 209 - DNA, 384 bp, Artificial Sequence
  synthetic
gaggtgcagctggtggagtctgggggaggcttggtacagcctggggggtccctgagactctcctgtgcagcctctggattcacctttagcaactatgccatgatctgggtccgccaggctccagggaaggggctggagtgggtctcaggtattagtggtagtggtggcagtatatactacgcagactccgtgaagggccggttcaccatctccagagacaattccaagaacacgctgtatctgcaaatgaacagcctgagagccgaggacacggccgtatattactgtgcgaaagaaggaattattagtatggttcggggacttatcaactactaccacggtatggacgtctggggccaagggaccacggtcaccgtctcctca

SEQ ID NO: 210 - protein, 128 aa, Artificial Sequence
  synthetic
EVQLVESGGGLVQPGGSLRLSCAASGFTFSNYAMIWVRQAPGKGLEWVSGISGSGGSIYYADSVKGRFTISRDNSKNTLYLQMNSLRAEDTAVYYCAKEGIISMVRGLINYYHGMDVWGQGTTVTVSS

SEQ ID NO: 211 - DNA, 24 bp, Artificial Sequence
  synthetic
ggattcacctttagcaactatgcc

SEQ ID NO: 212 - protein, 8 aa, Artificial Sequence
  synthetic
GFTFSNYA

SEQ ID NO: 213 - DNA, 24 bp, Artificial Sequence
  synthetic
attagtggtagtggtggcagtata

SEQ ID NO: 214 - protein, 8 aa, Artificial Sequence
  synthetic
ISGSGGSI

SEQ ID NO: 215 - DNA, 63 bp, Artificial Sequence
  synthetic
gcgaaagaaggaattattagtatggttcggggacttatcaactactaccacggtatggacgtc

SEQ ID NO: 216 - protein, 21 aa, Artificial Sequence
  synthetic
AKEGIISMVRGLINYYHGMDV

SEQ ID NO: 217 - DNA, 324 bp, Artificial Sequence
  synthetic
gaaattgtgttgacgcagtctccaggcaccctgtctttgtctccaggggaaagagccaccctctcctgcagggccagtcagagtgttagcagcagctacttagcctggtaccagcagaaacctggccaggctcccaggctcctcatctatggtgcatccagcagggccactggcatcccagacaggttcagtggcagtgggtctgggacagacttcactctcaccatcagcagactggagcctgaagattttgcagtgtattactgtcagcagtatggtagctcaccttggacgttcggccaagggaccaaggtggaaatcaaa

SEQ ID NO: 218 - protein, 108 aa, Artificial Sequence
  synthetic
EIVLTQSPGTLSLSPGERATLSCRASQSVSSSYLAWYQQKPGQAPRLLIYGASSRATGIPDRFSGSGSGTDFTLTISRLEPEDFAVYYCQQYGSSPWTFGQGTKVEIK

SEQ ID NO: 219 - DNA, 21 bp, Artificial Sequence
  synthetic
cagagtgttagcagcagctac

SEQ ID NO: 220 - protein, 7 aa, Artificial Sequence
  synthetic
QSVSSSY

SEQ ID NO: 221 - DNA, 9 bp, Artificial Sequence
  synthetic
ggtgcatcc

SEQ ID NO: 222 - protein, 3 aa, Artificial Sequence
  synthetic
GAS

SEQ ID NO: 223 - DNA, 27 bp, Artificial Sequence
  synthetic
cagcagtatggtagctcaccttggacg

SEQ ID NO: 224 - protein, 9 aa, Artificial Sequence
  synthetic
QQYGSSPWT

SEQ ID NO: 225 - DNA, 360 bp, Artificial Sequence
  synthetic
caggtgcagctggtgcagtctggggctgaggtgaagaagcctggggcctcagtgaaggtttcctgcaaggcatctggatacaccttcaccagctactatatgcactgggtgcgacaggcccctggacaagggcttgagtggttgggaataatcaaccctagtggtggtagcacaagctacgcacagaagttccagggcagagtcaccatgaccagggacacgtccacgagcacagtctacatggagctgagcagcctgagatctgaggacacggccgtgtattactgtgcgagagagacaggagaagctggtgaggtttttaactactggggccagggaacccaggtcaccgtctcctca

SEQ ID NO: 226 - protein, 120 aa, Artificial Sequence
  synthetic
QVQLVQSGAEVKKPGASVKVSCKASGYTFTSYYMHWVRQAPGQGLEWLGIINPSGGSTSYAQKFQGRVTMTRDTSTSTVYMELSSLRSEDTAVYYCARETGEAGEVFNYWGQGTQVTVSS

SEQ ID NO: 227 - DNA, 24 bp, Artificial Sequence
  synthetic
ggatacaccttcaccagctactat

SEQ ID NO: 228 - protein, 8 aa, Artificial Sequence
  synthetic
GYTFTSYY

SEQ ID NO: 229 - DNA, 24 bp, Artificial Sequence
  synthetic
atcaaccctagtggtggtagcaca

SEQ ID NO: 230 - protein, 8 aa, Artificial Sequence
  synthetic
INPSGGST

SEQ ID NO: 231 - DNA, 39 bp, Artificial Sequence
  synthetic
gcgagagagacaggagaagctggtgaggtttttaactac

SEQ ID NO: 232 - protein, 13 aa, Artificial Sequence
  synthetic
ARETGEAGEVFNY

SEQ ID NO: 233 - DNA, 324 bp, Artificial Sequence
  synthetic
gacatccagatgacccagtctccatcctccctgtctgcatctgtaggagacagagtcaccatcacttgccgggcaagtcagatcattagcaggtatttaaattggtatcagcataaaccagggaaagcccctaaggtcctgatctatgctgcctccactttgcaaagtggggtcccatcaaggttcagtggcagtggatctgggacagatttcactctcaccatcagcagtctgcaacctgaagattttgcaacttactactgtcaacagagttacagtacccctccgatcaccttcggccaagggacacgactggagattaaa

SEQ ID NO: 234 - protein, 108 aa, Artificial Sequence
  synthetic
DIQMTQSPSSLSASVGDRVTITCRASQIISRYLNWYQHKPGKAPKVLIYAASTLQSGVPSRFSGSGSGTDFTLTISSLQPEDFATYYCQQSYSTPPITFGQGTRLEIK

SEQ ID NO: 235 - DNA, 18 bp, Artificial Sequence
  synthetic
cagatcattagcaggtat

SEQ ID NO: 236 - protein, 6 aa, Artificial Sequence
  synthetic
QIISRY

SEQ ID NO: 237 - DNA, 9 bp, Artificial Sequence
  synthetic
gctgcctcc

SEQ ID NO: 238 - protein, 3 aa, Artificial Sequence
  synthetic
AAS

SEQ ID NO: 239 - DNA, 30 bp, Artificial Sequence
  synthetic
caacagagttacagtacccctccgatcacc

SEQ ID NO: 240 - protein, 10 aa, Artificial Sequence
  synthetic
QQSYSTPPIT

SEQ ID NO: 241 - DNA, 381 bp, Artificial Sequence
  synthetic
gaggtgcagctggtggagtctgggggaggcttggtacagcctggagggtccctgagactctcctgtgcagcctctggattcaccttcagtagttatgaaatgaactgggtccgccaggctccagggaaggggctggagtgggtttcatacattggtagtagtggtcgtgccacatactacgcagactctgtgaagggccgattcaccatctccagagacaacgccaaaaactcactgtatctgcaaatgaacagcctgagagccgaggacacggctgtttattactgtgcgagaccttcgagcatagcagctctgttacggaaccagtaccacttcggtatggacgtctggggccaagggaccacggtcaccgtctcctca

SEQ ID NO: 242 - protein, 127 aa, Artificial Sequence
  synthetic
EVQLVESGGGLVQPGGSLRLSCAASGFTFSSYEMNWVRQAPGKGLEWVSYIGSSGRATYYADSVKGRFTISRDNAKNSLYLQMNSLRAEDTAVYYCARPSSIAALLRNQYHFGMDVWGQGTTVTVSS

SEQ ID NO: 243 - DNA, 24 bp, Artificial Sequence
  synthetic
ggattcaccttcagtagttatgaa

SEQ ID NO: 244 - protein, 8 aa, Artificial Sequence
  synthetic
GFTFSSYE

SEQ ID NO: 245 - DNA, 24 bp, Artificial Sequence
  synthetic
attggtagtagtggtcgtgccaca

SEQ ID NO: 246 - protein, 8 aa, Artificial Sequence
  synthetic
IGSSGRAT

SEQ ID NO: 247 - DNA, 60 bp, Artificial Sequence
  synthetic
gcgagaccttcgagcatagcagctctgttacggaaccagtaccacttcggtatggacgtc

SEQ ID NO: 248 - protein, 20 aa, Artificial Sequence
  synthetic
ARPSSIAALLRNQYHFGMDV

SEQ ID NO: 249 - DNA, 324 bp, Artificial Sequence
  synthetic
gacatccagatgacccagtctccatcctccctgtctgcatctgtaggagacagagtcaccatcacttgccgggcaagtcagagcattaccagctatttaaattggtatcagcagaaaccagggaaagcccctaagctcctgatctatgctgcatccagtttgcaaggtggggtcccatcaaggttcagtggcagtggatctgggacagatttcactctcaccatcagcagtctgcaacctgaagattttgcaacttactactgtcaacagagttacagtacccctccgatcaccttcggccaagggacacgactggagattaaa

SEQ ID NO: 250 - protein, 108 aa, Artificial Sequence
  synthetic
DIQMTQSPSSLSASVGDRVTITCRASQSITSYLNWYQQKPGKAPKLLIYAASSLQGGVPSRFSGSGSGTDFTLTISSLQPEDFATYYCQQSYSTPPITFGQGTRLEIK

SEQ ID NO: 251 - DNA, 18 bp, Artificial Sequence
  synthetic
cagagcattaccagctat

SEQ ID NO: 252 - protein, 6 aa, Artificial Sequence
  synthetic
QSITSY

SEQ ID NO: 253 - DNA, 9 bp, Artificial Sequence
  synthetic
gctgcatcc

SEQ ID NO: 254 - protein, 3 aa, Artificial Sequence
  synthetic
AAS

SEQ ID NO: 255 - DNA, 30 bp, Artificial Sequence; identical to SEQ ID NO: 239
  synthetic

SEQ ID NO: 256 - protein, 10 aa, Artificial Sequence
  synthetic
QQSYSTPPIT

SEQ ID NO: 257 - DNA, 360 bp, Artificial Sequence
  synthetic
caggtgcagctggtgcagtctggggctgaggtgaagaagcctggggcctcagtgaaggtttcctgcaaggcatctggatacaccttcaccagctactatatgcactgggtgcgacaggcccctggacaagggcttgagtggatgggaataatcaaccctagtggtggtagcacaagctacgcacagaagttccagggcagagtcaccatgaccagggacacgtccacgagcacagtctacatggagctgagcagcctgagatctgaggacacggccgtgtattactgtgcgagagagataggagaagctggtgaagtttttaactactggggccagggaaccctggtcaccgtctcctca

SEQ ID NO: 258 - protein, 120 aa, Artificial Sequence
  synthetic
QVQLVQSGAEVKKPGASVKVSCKASGYTFTSYYMHWVRQAPGQGLEWMGIINPSGGSTSYAQKFQGRVTMTRDTSTSTVYMELSSLRSEDTAVYYCAREIGEAGEVFNYWGQGTLVTVSS

SEQ ID NO: 259 - DNA, 24 bp, Artificial Sequence
  synthetic
ggatacaccttcaccagctactat

SEQ ID NO: 260 - protein, 8 aa, Artificial Sequence
  synthetic
GYTFTSYY

SEQ ID NO: 261 - DNA, 24 bp, Artificial Sequence
  synthetic
atcaaccctagtggtggtagcaca

SEQ ID NO: 262 - protein, 8 aa, Artificial Sequence
  synthetic
INPSGGST

SEQ ID NO: 263 - DNA, 39 bp, Artificial Sequence
  synthetic
gcgagagagataggagaagctggtgaagtttttaactac

SEQ ID NO: 264 - protein, 13 aa, Artificial Sequence
  synthetic
AREIGEAGEVFNY

SEQ ID NO: 265 - DNA, 324 bp, Artificial Sequence
  synthetic
gacatccagatgacccagtctccatcctccctgtctgcatctgtaggagacagagtcaccatcacttgccgggcaagtcagagcattagcaggtatttaaattggtatcagcataaaccagggaaagcccctaaggtcctgatctatgctgcatccattttgcaaagtggggtcccatcaaggttcagtggcagtggatctgggacagatttcactctcaccatcagcagtctgcaacctgaagattttgcaacttactactgtcaacagagttacagtacccctccgatcaccttcggccaagggacacgactggagattaaa

SEQ ID NO: 266 - protein, 108 aa, Artificial Sequence
  synthetic
DIQMTQSPSSLSASVGDRVTITCRASQSISRYLNWYQHKPGKAPKVLIYAASILQSGVPSRFSGSGSGTDFTLTISSLQPEDFATYYCQQSYSTPPITFGQGTRLEIK

SEQ ID NO: 267 - DNA, 18 bp, Artificial Sequence
  synthetic
cagagcattagcaggtat

SEQ ID NO: 268 - protein, 6 aa, Artificial Sequence
  synthetic
QSISRY

SEQ ID NO: 269 - DNA, 9 bp, Artificial Sequence
  synthetic
gctgcatcc

SEQ ID NO: 270 - protein, 3 aa, Artificial Sequence
  synthetic
AAS

SEQ ID NO: 271 - DNA, 30 bp, Artificial Sequence; identical to SEQ ID NO: 239
  synthetic

SEQ ID NO: 272 - protein, 10 aa, Artificial Sequence
  synthetic
QQSYSTPPIT

SEQ ID NO: 273 - DNA, 381 bp, Artificial Sequence
  synthetic
gaggtgcagctggtggagtctgggggaggcttggtacagcctggagggtccctgagactctcctgtgcagcctctggattcaccttcagtacttatgaaatgaactgggtccgccaggctccagggaaggggctggagtgggtttcatatagtagtagtagtggtagaaccatatactacgcagactctgtgaagggccgattcaccatctccagagacaacgccaagaactcactgtttctgcaaatgaacagcctgagagccgaggacacggctgtttattactgtgcgagaccttcgagtatagagactctgttacggaatcagtaccactacggtgtggacgtctggggccaagggaccacggtcaccgtctcctca

SEQ ID NO: 274 - protein, 127 aa, Artificial Sequence
  synthetic
EVQLVESGGGLVQPGGSLRLSCAASGFTFSTYEMNWVRQAPGKGLEWVSYSSSSGRTIYYADSVKGRFTISRDNAKNSLFLQMNSLRAEDTAVYYCARPSSIETLLRNQYHYGVDVWGQGTTVTVSS

SEQ ID NO: 275 - DNA, 24 bp, Artificial Sequence
  synthetic
ggattcaccttcagtacttatgaa

SEQ ID NO: 276 - protein, 8 aa, Artificial Sequence
  synthetic
GFTFSTYE

SEQ ID NO: 277 - DNA, 24 bp, Artificial Sequence
  synthetic
agtagtagtagtggtagaaccata

SEQ ID NO: 278 - protein, 8 aa, Artificial Sequence
  synthetic
SSSSGRTI

SEQ ID NO: 279 - DNA, 60 bp, Artificial Sequence
  synthetic
gcgagaccttcgagtatagagactctgttacggaatcagtaccactacggtgtggacgtc

SEQ ID NO: 280 - protein, 20 aa, Artificial Sequence
  synthetic
ARPSSIETLLRNQYHYGVDV

SEQ ID NO: 281 - DNA, 324 bp, Artificial Sequence
  synthetic
gacatccagatgacccagtctccatcctccctgtctgcatctgtaggagacagagtcaccatcacttgccgggcaagtcagagcattagcagctatttaaattggtatcagcagaaaccagggaaagcccctaagctcctgatctatgctgcatccagtttgcaaagtggggtcccgtcaaggttcagtggcagtggatctgggacagatttcactctcaccatcagcagtctgcaacctgaagattttgcaacttactactgtcaacagagttacagtacccctccgatcaccttcggccaagggacacgactggagattaaa

SEQ ID NO: 282 - protein, 108 aa, Artificial Sequence
  synthetic
DIQMTQSPSSLSASVGDRVTITCRASQSISSYLNWYQQKPGKAPKLLIYAASSLQSGVPSRFSGSGSGTDFTLTISSLQPEDFATYYCQQSYSTPPITFGQGTRLEIK

SEQ ID NO: 283 - DNA, 18 bp, Artificial Sequence
  synthetic
cagagcattagcagctat

SEQ ID NO: 284 - protein, 6 aa, Artificial Sequence
  synthetic
QSISSY

SEQ ID NO: 285 - DNA, 9 bp, Artificial Sequence
  synthetic
gctgcatcc

SEQ ID NO: 286 - protein, 3 aa, Artificial Sequence
  synthetic
AAS

SEQ ID NO: 287 - DNA, 30 bp, Artificial Sequence; identical to SEQ ID NO: 239
  synthetic

SEQ ID NO: 288 - protein, 10 aa, Artificial Sequence
  synthetic
QQSYSTPPIT

SEQ ID NO: 289 - DNA, 384 bp, Artificial Sequence
  synthetic
gaggtgcagctggtggagtctgggggaggcttggcacagcctggagggtccctgagactctcctgtgcagcctctggattcaccttcagtagtcatgaaatgaactgggtccgccaggctccagggaaggggctggagtgggtttcatacattagtcgtagtggtagaatcataaactacgcagactctgtgaagggccgattcaccatctccagagacaacgccaagaactcactgtatctgcaaatgaacagcctgagagccgaggacacggctgtttattactgtgcgagagagagaggctcgtattacgatattttgactggttcccaggactacggtatggacgtctggggccaagggaccacggtcaccgtctcctca

SEQ ID NO: 290 - protein, 128 aa, Artificial Sequence
  synthetic
EVQLVESGGGLAQPGGSLRLSCAASGFTFSSHEMNWVRQAPGKGLEWVSYISRSGRIINYADSVKGRFTISRDNAKNSLYLQMNSLRAEDTAVYYCARERGSYYDILTGSQDYGMDVWGQGTTVTVSS

SEQ ID NO: 291 - DNA, 24 bp, Artificial Sequence
  synthetic
ggattcaccttcagtagtcatgaa

SEQ ID NO: 292 - protein, 8 aa, Artificial Sequence
  synthetic
GFTFSSHE

SEQ ID NO: 293 - DNA, 24 bp, Artificial Sequence
  synthetic
attagtcgtagtggtagaatcata

SEQ ID NO: 294 - protein, 8 aa, Artificial Sequence
  synthetic
ISRSGRII

SEQ ID NO: 295 - DNA, 63 bp, Artificial Sequence
  synthetic
gcgagagagagaggctcgtattacgatattttgactggttcccaggactacggtatggacgtc

SEQ ID NO: 296 - protein, 21 aa, Artificial Sequence
  synthetic
ARERGSYYDILTGSQDYGMDV

SEQ ID NO: 297 - DNA, 324 bp, Artificial Sequence
  synthetic
gacatccagatgacccagtctccatcctccctgtctgcatctgtaggagacagagtcaccatcacttgccgggcaagtcagaccattagcacctatttaaattggtatcagcagaaaccagggaaagcccctaagctcctgatctatgctgcatccagtttgcaaagtggggtcccatcaaggttcagtggcagtggatctgggacagatttcactctcaccatcagcagtctgcaacctgaagattttgcaacttactactgtcaacagagttacagtacccctccgatcaccttcggccaagggacacgactggagattaaa

SEQ ID NO: 298 - protein, 108 aa, Artificial Sequence
  synthetic
DIQMTQSPSSLSASVGDRVTITCRASQTISTYLNWYQQKPGKAPKLLIYAASSLQSGVPSRFSGSGSGTDFTLTISSLQPEDFATYYCQQSYSTPPITFGQGTRLEIK

SEQ ID NO: 299 - DNA, 18 bp, Artificial Sequence
  synthetic
cagaccattagcacctat

SEQ ID NO: 300 - protein, 6 aa, Artificial Sequence
  synthetic
QTISTY

SEQ ID NO: 301 - DNA, 9 bp, Artificial Sequence
  synthetic
gctgcatcc

SEQ ID NO: 302 - protein, 3 aa, Artificial Sequence
  synthetic
AAS

SEQ ID NO: 303 - DNA, 30 bp, Artificial Sequence; identical to SEQ ID NO: 239
  synthetic

SEQ ID NO: 304 - protein, 10 aa, Artificial Sequence
  synthetic
QQSYSTPPIT

SEQ ID NO: 305 - DNA, 381 bp, Artificial Sequence
  synthetic
gaggtgcagctggtggagtctgggggaggcttggtacagcctggagggtccctgagactctcctgtgcagcctctggattcaccttcagtagttatgaaatgaactgggtccgccaggctccagggaaggggctggagtgggtttcatacattagtagtagtggtagtaccaaatactacgcagactctgtgaagggccgattcaccatctccagagacaacgccaagaactcactgtatctgcaaatgaacagcctgagagccgaggacacggctgtttattactgtgcgagaccttcgagtataccagctctgttacggaaccagtaccactacggtatggacgtctggggccaagggaccacggtcaccgtctcctca

SEQ ID NO: 306 - protein, 127 aa, Artificial Sequence
  synthetic
EVQLVESGGGLVQPGGSLRLSCAASGFTFSSYEMNWVRQAPGKGLEWVSYISSSGSTKYYADSVKGRFTISRDNAKNSLYLQMNSLRAEDTAVYYCARPSSIPALLRNQYHYGMDVWGQGTTVTVSS

SEQ ID NO: 307 - DNA, 24 bp, Artificial Sequence
  synthetic
ggattcaccttcagtagttatgaa

SEQ ID NO: 308 - protein, 8 aa, Artificial Sequence
  synthetic
GFTFSSYE

SEQ ID NO: 309 - DNA, 24 bp, Artificial Sequence
  synthetic
attagtagtagtggtagtaccaaa

SEQ ID NO: 310 - protein, 8 aa, Artificial Sequence
  synthetic
ISSSGSTK

SEQ ID NO: 311 - DNA, 60 bp, Artificial Sequence
  synthetic
gcgagaccttcgagtataccagctctgttacggaaccagtaccactacggtatggacgtc

SEQ ID NO: 312 - protein, 20 aa, Artificial Sequence
  synthetic
ARPSSIPALLRNQYHYGMDV

SEQ ID NO: 313 - DNA, 2051 bp, Ebola virus
gaattcgccaccatgggcgtgaccggcatcctgcagctgccccgggacagattcaagcggaccagcttcttcctgtgggtcatcatcctgttccagcggaccttcagcatccccctgggcgtgatccacaacagcaccctgcaggtgtccgacgtggacaagctcgtgtgccgggacaagctgagcagcaccaaccagctgagaagcgtgggcctgaacctggaaggcaatggcgtggccaccgatgtgcctagcgccaccaagagatggggcttcagatccggcgtgccccccaaggtcgtgaattatgaggccggcgagtgggccgagaactgctacaacctggaaatcaagaagcccgacggcagcgagtgcctgcctgctgcccctgatggcatcagaggcttcccccggtgcagatacgtgcacaaggtgtccggcacaggcccctgcgctggcgatttcgcctttcacaaagagggcgcctttttcctgtacgaccggctggcctccaccgtgatctacagaggcaccacctttgccgagggcgtggtggcctttctgatcctgcctcaggccaagaaggacttcttcagcagccaccccctgcgcgagcctgtgaatgccacagaggatcccagcagcggctactacagcaccaccatcagataccaggccaccggcttcggcaccaacgagacagagtacctgttcgaggtggacaacctgacctacgtgcagctggaaagccggttcaccccccagtttctgctgcagctgaacgagacaatctacgccagcggcaagcggagcaacaccaccggcaagctgatctggaaagtgaaccccgagatcgataccacaatcggagagtgggccttctgggagacaaagaagaacctgacccggaagatcagaagcgaggaactgagcttcaccgccgtgtccaacggccccaagaacatcagcggacagagccccgccagaaccagcagcgaccccgagacaaacaccaccaatgaggaccacaagatcatggccagcgagaacagcagcgccatggtgcaggtgcacagccagggaagaaaggccgctgtgtcccacctgaccaccctggccacaatctccaccagccctcagagcctgaccacaaagcctggccccgacaactccacccacaacacccccgtgtacaagctggacatcagcgaggccacacaagtgggccagcaccacagaagggccgacaacgatagcaccgccagcgatacccctccagccacaactgctgccggacctctgaaggccgagaataccaacaccagcaagagcgccgacagcctggatctggccaccaccacaagcccccagaactactctgagacagccggcaacaacaacacccaccaccaggataccggcgaggaaagcgccagctctggcaagctgggactgatcaccaacacaatcgccggcgtggccggcctgattaccggggggagaagaaccagacgggaagtgatcgtgaacgcccagcccaagtgcaaccccaacctgcactactggaccacccaggatgagggcgctgctatcggactggcctggatcccttactttggccctgccgccgagggcatctacaccgagggactgatgcacaaccaggacggcctgatctgcggactgaggcagctggccaacgaaaccacacaggctctgcagctgttcctgagagccaccaccgagctgaggaccttctccatcctgaacagaaaggctatcgacttcctgctgcagcgctggggcggcacctgtcacattctgggccctgactgctgcatcgagccccacgactggaccaagaatatcaccgacaagatcgaccagatcatccacgactttgtggacaagaccctgcccgaccagggcgacaatgacaactggtggacaggctggcggcagtggattcctgccggcattggagtgaccggcgtgatcattgccgtgatcgccctgttctgcatctgcaagttcgtgttctgagcggccgc

SEQ ID NO: 314 - protein, 676 aa, Ebola virus
MGVTGILQLPRDRFKRTSFFLWVIILFQRTFSIPLGVIHNSTLQVSDVDKLVCRDKLSSTNQLRSVGLNLEGNGVATDVPSATKRWGFRSGVPPKVVNYEAGEWAENCYNLEIKKPDGSECLPAAPDGIRGFPRCRYVHKVSGTGPCAGDFAFHKEGAFFLYDRLASTVIYRGTTFAEGVVAFLILPQAKKDFFSSHPLREPVNATEDPSSGYYSTTIRYQATGFGTNETEYLFEVDNLTYVQLESRFTPQFLLQLNETIYASGKRSNTTGKLIWKVNPEIDTTIGEWAFWETKKNLTRKIRSEELSFTAVSNGPKNISGQSPARTSSDPETNTTNEDHKIMASENSSAMVQVHSQGRKAAVSHLTTLATISTSPQPPTTKTGPDNSTHNTPVYKLDISEATQVGQHHRRADNDSTASDTPPATTAAGPLKAENTNTSKSADSLDLATTTSPQNYSETAGNNNTHHQDTGEESASSGKLGLITNTIAGVAGLITGGRRTRREVIVNAQPKCNPNLHYWTTQDEGAAIGLAWIPYFGPAAEGIYTEGLMHNQDGLICGLRQLANETTQALQLFLRATTELRTFSILNRKAIDFLLQRWGGTCHILGPDCCIEPHDWTKNITDKIDQIIHDFVDKTLPDQGDNDNWWTGWRQWIPAGIGVTGVIIAVIALFCICKFVF

SEQ ID NO: 315 - protein, 676 aa, Ebola virus; identical to SEQ ID NO: 314

SEQ ID NO: 316 - protein, 364 aa, Ebola virus
MGVTGILQLPRDRFKRTSFFLWVIILFQRTFSIPLGVIHNSTLQVSDVDKLVCRDKLSSTNQLRSVGLNLEGNGVATDVPSATKRWGFRSGVPPKVVNYEAGEWAENCYNLEIKKPDGSECLPAAPDGIRGFPRCRYVHKVSGTGPCAGDFAFHKEGAFFLYDRLASTVIYRGTTFAEGVVAFLILPQAKKDFFSSHPLREPVNATEDPSSGYYSTTIRYQATGFGTNETEYLFEVDNLTYVQLESRFTPQFLLQLNETIYASGKRSNTTGKLIWKVNPEIDTTIGEWAFWETKKTSLEKFAVKSCLSQLYQTDPKTSVVRVRRELLPTQRPTQQMKTTKSWLQKIPLQWFKCTVKEGKLQCRI

SEQ ID NO: 317 - protein, 360 aa, Artificial Sequence
  aa 1-332: Zaire_Ebola_GP aa 33 through 364 of AHX24650 aa 333-360: myc-myc-hexahistidine tag
IPLGVIHNSTLQVSDVDKLVCRDKLSSTNQLRSVGLNLEGNGVATDVPSATKRWGFRSGVPPKVVNYEAGEWAENCYNLEIKKPDGSECLPAAPDGIRGFPRCRYVHKVSGTGPCAGDFAFHKEGAFFLYDRLASTVIYRGTTFAEGVVAFLILPQAKKDFFSSHPLREPVNATEDPSSGYYSTTIRYQATGFGTNETEYLFEVDNLTYVQLESRFTPQFLLQLNETIYASGKRSNTTGKLIWKVNPEIDTTIGEWAFWETKKTSLEKFAVKSCLSQLYQTDPKTSVVRVRRELLPTQRPTQQMKTTKSWLQKIPLQWFKCTVKEGKLQCRIEQKLISEEDLGGEQKLISEEDLHHHHHH

SEQ ID NO: 318 - protein, 628 aa, Artificial Sequence
  aa 1-618: Zaire ebolavirus (strain H.sapiens-wt/GIN/2014/Kissidougou-C15) GP (aa 33 through 650  (AHX24649.1)) aa 619-628: decahistidine tag
IPLGVIHNSTLQVSDVDKLVCRDKLSSTNQLRSVGLNLEGNGVATDVPSATKRWGFRSGVPPKVVNYEAGEWAENCYNLEIKKPDGSECLPAAPDGIRGFPRCRYVHKVSGTGPCAGDFAFHKEGAFFLYDRLASTVIYRGTTFAEGVVAFLILPQAKKDFFSSHPLREPVNATEDPSSGYYSTTIRYQATGFGTNETEYLFEVDNLTYVQLESRFTPQFLLQLNETIYTSGKRSNTTGKLIWKVNPEIDTTIGEWAFWETKKNLTRKIRSEELSFTVVSNGAKNISGQSPARTSSDPGTNTTTEDHKIMASENSSAMVQVHSQGREAAVSHLTTLATISTSPQSLTTKPGPDNSTHNTPVYKLDISEATQVEQHHRRTDNDSTASDTPSATTAAGPPKAENTNTSKSTDFLDPATTTSPQNHSETAGNNNTHHQDTGEESASSGKLGLITNTIAGVAGLITGGRRTRREAIVNAQPKCNPNLHYWTTQDEGAAIGLAWIPYFGPAAEGIYIEGLMHNQDGLICGLRQLANETTQALQLFLRATTELRTFSILNRKAIDFLLQRWGGTCHILGPDCCIEPHDWTKNITDKIDQIIHDFVDKTLPDQGDNDNWWTGWRQHHHHHHHHHH